European Patent Specification EP 3 620 470 B1, published July 26, 2023. Title: TEM8 ANTIBODIES AND THEIR USE. Applicant: The United States of America as Represented by the Secretary, Department of Health and Human Services BioMed Valley Discoveries, Inc. Dimitrov, Dimiter Zhu, Zhongyu St. Croix, Brad Zudaire, Enrique Saha, Saurabh Zhang, Xiaoyan DeCrescenzo, Gary Welsch, Dean. The sequence listing filed with the application follows.

SEQUENCE LISTING (28 sequences)

SEQ ID NO: 1 - protein, 117 aa, Artificial Sequence
  antibody sequence
QVQLVQSGAEVKKPGTSVKVSCKVPGYTFSSYAISWVRQAPGQGLEWMGGIIPIFGTTNYAQKFQGRVTITGEESTSTVYMELSSLRSEDTAVYYCARDTDYMFDYWGQGTLVTVSS

SEQ ID NO: 2 - protein, 107 aa, Artificial Sequence [sequence omitted]

SEQ ID NO: 3 - protein, 117 aa, Artificial Sequence
  antibody sequence
QVQLVQSGAEVKKPGASVKVSCKVSGYTFSSYAISWVRQAPGQGLEWMGGIIPIFGTANYAQKFQGRVTITADESTSTAYMELSSLRSEDTAVYYCARDTDYMFDYWGQGTLVTVSS

SEQ ID NO: 4 - protein, 107 aa, Artificial Sequence [sequence omitted]

SEQ ID NO: 5 - protein, 121 aa, Artificial Sequence
  antibody sequence
EVQLVESGGGVVQPGRSVRLSCAASGFTFSTYTMHWVRQAPGKGLEWVAIISNDGSNKYYADPVRGRFTISRDNSKNTLYLQMNSLRAEDTAVYYCVRGSSWYRGNWFDPWGQGTLVTVSS

SEQ ID NO: 6 - protein, 108 aa, Artificial Sequence
  antibody sequence
DIQMTQSPSSLSASVGDRVTIACRASQTISRYLNWYQQKPGKAPKLLIYAASSLQSGVSSRFSGSGSGTEFTLTISSLQPEDFATYFCQQTYSPPITFGQGTRLEIKR

SEQ ID NO: 7 - protein, 121 aa, Artificial Seuqence
  antibody sequence
EVQLVETGAEVKKPGASVKVSCKASGYTFTGYYMHWVRQAPGQGLEWMGWINPTSGSTNYAQKFQGRVTMTRDTSISTAYMELSGLRSDDTAVYYCVRDPGSPKWLAFDPWGQGTLVTVSS

SEQ ID NO: 8 - protein, 108 aa, Artificial Sequence
  antibody sequence
DIQLTQSPSSLSASVGDRVTITCRASRAISRYLNWYQQKPGKAPKLLIYAASSLQSGVSSRFSGSGSGTEFTLTISSLQPEDFATYFCQQTYSPPITFGQGTRLEIKR

SEQ ID NO: 9 - DNA, 1695 bp, Homo sapiens
atggccacggcggagcggagagccctcggcatcggcttccagtggctctctttggccactctggtgctcatctgcgccgggcaagggggacgcagggaggatgggggtccagcctgctacggcggatttgacctgtacttcattttggacaaatcaggaagtgtgctgcaccactggaatgaaatctattactttgtggaacagttggctcacaaattcatcagcccacagttgagaatgtcctttattgttttctccacccgaggaacaaccttaatgaaactgacagaagacagagaacaaatccgtcaaggcctagaagaactccagaaagttctgccaggaggagacacttacatgcatgaaggatttgaaagggccagtgagcagatttattatgaaaacagacaagggtacaggacagccagcgtcatcattgctttgactgatggagaactccatgaagatctctttttctattcagagagggaggctaataggtctcgagatcttggtgcaattgtttactgtgttggtgtgaaagatttcaatgagacacagctggcccggattgcggacagtaaggatcatgtgtttcccgtgaatgacggctttcaggctctgcaaggcatcatccactcaattttgaagaagtcctgcatcgaaattctagcagctgaaccatccaccatatgtgcaggagagtcatttcaagttgtcgtgagaggaaacggcttccgacatgcccgcaacgtggacagggtcctctgcagcttcaagatcaatgactcggtcacactcaatgagaagcccttttctgtggaagatacttatttactgtgtccagcgcctatcttaaaagaagttggcatgaaagctgcactccaggtcagcatgaacgatggcctctcttttatctccagttctgtcatcatcaccaccacacactgttctgacggttccatcctggccatcgccctgctgatcctgttcctgctcctagccctggctctcctctggtggttctggcccctctgctgcactgtgattatcaaggaggtccctccaccccctgccgaggagagtgaggaagaagatgatgatggtctgcctaagaaaaagtggccaacggtagacgcctcttattatggtgggagaggcgttggaggcattaaaagaatggaggttcgttggggagaaaagggctccacagaagaaggtgctaagttggaaaaggcaaagaatgcaagagtcaagatgccggagcaggaatatgaattccctgagccgcgaaatctcaacaacaatatgcgtcggccttcttccccccggaagtggtactctccaatcaagggaaaactcgatgccttgtgggtcctactgaggaaaggatatgatcgtgtgtctgtgatgcgtccacagccaggagacacggggcgctgcatcaacttcaccagggtcaagaacaaccagccagccaagtacccactcaacaacgcctaccacacctcctcgccgcctcctgcccccatctacactcccccacctcctgcgccccactgccctcccccgccccccagcgcccctacccctcccatcccgtccccaccttccacccttccccctcctccccaggctccacctcccaacagggcacctcctccctcccgccctcctccaaggccttctgtctag

SEQ ID NO: 10 - protein, 564 aa, Homo sapiens
MATAERRALGIGFQWLSLATLVLICAGQGGRREDGGPACYGGFDLYFILDKSGSVLHHWNEIYYFVEQLAHKFISPQLRMSFIVFSTRGTTLMKLTEDREQIRQGLEELQKVLPGGDTYMHEGFERASEQIYYENRQGYRTASVIIALTDGELHEDLFFYSEREANRSRDLGAIVYCVGVKDFNETQLARIADSKDHVFPVNDGFQALQGIIHSILKKSCIEILAAEPSTICAGESFQVVVRGNGFRHARNVDRVLCSFKINDSVTLNEKPFSVEDTYLLCPAPILKEVGMKAALQVSMNDGLSFISSSVIITTTHCSDGSILAIALLILFLLLALALLWWFWPLCCTVIIKEVPPPPAEESEEEDDDGLPKKKWPTVDASYYGGRGVGGIKRMEVRWGEKGSTEEGAKLEKAKNARVKMPEQEYEFPEPRNLNNNMRRPSSPRKWYSPIKGKLDALWVLLRKGYDRVSVMRPQPGDTGRCINFTRVKNNQPAKYPLNNAYHTSSPPPAPIYTPPPPAPHCPPPPPSAPTPPIPSPPSTLPPPPQAPPPNRAPPPSRPPPRPSV

SEQ ID NO: 11 - DNA, 351 bp, Artificial Sequence
  antibody sequence
caggtccagctggtgcagtctggggctgaggtgaagaagcctgggacctcagtgaaggtctcctgcaaggttcctggatacaccttcagcagctatgctatcagctgggtgcgacaggcccctggacaagggcttgagtggatgggagggatcatccctatctttggtacaacaaactacgcacagaagttccagggcagagtcacgattaccggggaggaatccacgagcacagtctacatggagctgagcagcctgagatctgaggacacggccgtgtattactgtgcgagagatacggactacatgtttgactactggggccagggaaccctggtcaccgtgagctca

SEQ ID NO: 12 - DNA, 321 bp, Artificial Sequence
  antibody sequence
tcttctgagctgactcaggaccctgttgtgtctgtggccttgggagagacagtcagtatcacatgccaaggagacaacctcagagacttttatgcaagctggtaccaacagaagccaggacaggcccctctactagtcatgtatggtaaaaacaggcggccctcagggatcccagaccgattctctggctccacctcaggaaacacactttccttgaccatcactggggctcaggcggaagatgaggctgactattactgtagctcccgggacaacagtaagcatgtggtgttcggcggggggaccaaggtcaccgtccta

SEQ ID NO: 13 - DNA, 351 bp, Artificial Sequence
  antibody sequence
caggtccagctggtgcagtctggggctgaggtgaagaagcctggggcctcagtgaaggtctcctgcaaggtttctggatacaccttcagcagctatgctatcagctgggtgcgacaggcccctggacaagggcttgagtggatgggagggatcatccctatctttggtacagcaaactacgcacagaagttccagggcagagtcacgattaccgcggacgaatccacgagcacagcctacatggagctgagcagcctgagatctgaggacacggccgtgtattactgtgcgagagatacggactacatgtttgactactggggccagggaaccctggtcaccgtgagctca

SEQ ID NO: 14 - DNA, 321 bp, Artificial sequence; identical to SEQ ID NO: 12
  antibody sequence

SEQ ID NO: 15 - DNA, 363 bp, Artificial Sequence
  antibody sequence
gaggtgcagctggtggagtctgggggaggcgtggtccagcctgggaggtccgtgagactctcctgtgcagcctctggattcaccttcagtacctatactatgcactgggtccgccaggctccaggcaaggggctggagtgggtggcaattatctcaaatgatggaagcaataagtactacgcagaccccgtgaggggccgattcaccatctccagagacaattccaagaacacgctgtatctgcaaatgaacagcctgagagctgaggacacggctgtgtattactgtgtacgtggcagcagctggtatcgcggaaattggttcgacccctggggccagggaaccctggtcaccgtgagctca

SEQ ID NO: 16 - DNA, 324 bp, Artificial Sequence
  antibody sequence
gacatccagatgacccagtctccatcctccctgtctgcatctgtaggagacagagtcaccatcgcttgccgggcaagtcagaccattagtaggtatttaaattggtatcagcagaaaccagggaaagcccctaagctcctgatctatgctgcatccagtttgcaaagtggggtctcatcaaggttcagtggcagtggatctgggacagagttcactctcaccatcagcagtctgcagcctgaagattttgcaacttatttctgtcaacagacttacagtcccccgatcaccttcggccaagggacacgactggagattaaacga

SEQ ID NO: 17 - DNA, 363 bp, Artificial Sequence
  antibody sequence
gaggtgcagctggtggagaccggggctgaggtgaagaagcctggggcctcagtgaaggtctcctgcaaggcttctggatacaccttcaccggctactatatgcactgggtgcgacaggcccctggacaagggcttgagtggatgggatggatcaaccctaccagtggtagcacaaactatgcacagaagtttcagggcagggtcaccatgaccagggacacgtccatcagcacagcctacatggagctgagcgggctgagatctgacgacactgccgtgtattactgtgtgagagatccgggttctcctaagtggctggccttcgacccctggggccagggcaccctggtcaccgtgagctca

SEQ ID NO: 18 - DNA, 324 bp, Artificial Sequence
  antibody sequence
gacatccagttgacccagtctccatcctccttgtctgcttctgtaggagacagagtcaccatcacttgccgggcaagtcgggccattagtaggtatttaaattggtatcagcagaaaccagggaaagcccctaagctcctgatctatgctgcatccagtttgcaaagtggggtctcatcaaggttcagtggcagtggatctgggacagagttcactctcaccatcagcagtctgcagcctgaagattttgcaacttatttctgtcaacagacttacagtcccccgatcaccttcggccaagggacacgactggagattaaacgt

SEQ ID NO: 19 - protein, 15 aa, Artificial Sequence
  Peptide linker
GGGGSGGGGSGGGGS

SEQ ID NO: 20 - protein, 22 aa, homo sapiens
LLVTSLLLCELPHPAFLLIPDT

SEQ ID NO: 21 - protein, 236 aa, homo sapiens
EPKSCDKTHTCPPCPAPELLGGPSVFLFPPKPKDTLMISRTPEVTCVVVDVSHEDPEVKFNWYVDGVEVHNAKTKPREEQYNSTYRVVSVLTVLHQDWLNGKEYKCKVSNKALPAPIEKTISKAKGQPREPQVYTLPPSRDELTKNQVSLTCLVKGFYPSDIAVEWESNGQPENNYKTTPPVLDSDGSFFLYSKLTVDKSRWQQGNVFSCSVMHEALHNHYTQKSLSLSPGKKDPK

SEQ ID NO: 22 - protein, 69 aa, homo sapiens
TTTPAPRPPTPAPTIASQPLSLRPEACRPAAGGAVHTRGLDFACDIYIWAPLAGTCGVLLLSLVITLYC

SEQ ID NO: 23 - protein, 67 aa, homo sapiens
IEVMYPPPYLDNEKSNGTIIHVKGKHLCPSPLFPGPSKPFWVLVVVGGVLACYSLLVTVAFIIFWVR

SEQ ID NO: 24 - protein, 112 aa, homo sapiens
RVKFSRSADAPAYQQGQNQLYNELNLGRREEYDVLDKRRGRDPEMGGKPRRKNPQEGLYNELQKDKMAEAYSEIGMKGERRRGKGHDGLYQGLSTATKDTYDALHMQALPPR

SEQ ID NO: 25 - protein, 84 aa, homo sapiens
FVPVFLPAKPTTTPAPRPPTPAPTIASQPLSLRPEACRPAAGGAVHTRGLDFACDIYIWAPLAGTCGVLLLSLVITLYCNHRNR

SEQ ID NO: 26 - protein, 40 aa, homo sapiens
SKRSRLLHSDYMNMTPRRPGPTRKHYQPYAPPRDFAAYRS

SEQ ID NO: 27 - protein, 42 aa, homo sapiens
KRGRKKLLYIFKQPFMRPVQTTQEEDGCSCRFPEEEEGGCEL

SEQ ID NO: 28 - protein, 47 aa, homo sapiens
RFSVVKRGRKKLLYIFKQPFMRPVQTTQEEDGCSCRFPEEEEGGCEL